European Patent Application EP 4 563 146 A1, published June 4, 2025. Title: Flavivirus Inhibitors. Applicant: IRBM S.p.A. Application EP, filed November 28, 2023. The sequence listing filed with the application follows.

SEQUENCE LISTING (7 sequences)

SEQ ID NO: 1 - protein, 247 aa, Zika virus
MGSSHHHHHHSSGLVPRGSHMVDMYIERAGDITWEKDAEVTGNSPRLDVALDESGDFSLVEDDGPPMAGGGGSGGGGSGALWDVPAPKEVKKGETTDGVYRVMTRGLLGSTQVGVGVMQEGVFHTMWHVTKGSALRSGEGRLDPYWGDVKQDLVSYCGPWKLDAAWDGHSEVQLLAVPPGERARNIQTLPGIFKTKDGDIGAVALDYPAGTSGSPILDKCGRVIGLYGNGVVIKNGSYVSAITQGRR

SEQ ID NO: 2 - protein, 262 aa, Dengue virus
MGSSHHHHHHSSGLVPRGSHMADLELERAADVRWEEQAEISGSSPILSITISEDGSMSIKNEEEEQTLGGGGSGGGGAGVLWDVPSPPPVGKAELEDGAYRIKQKGILGYSQIGAGVYKEGTFHTMWHVTRGAVLMHKGKRIEPSWADVKKDLISYGGGWKLEGEWKEGEEVQVLALEPGKNPRAVQTKPGLFKTNTGTIGAVSLDFSPGTSGSPIVDKKGKVVGLYGNGVVTRSGAYVSAIAQTEKSIEDNPEIEDDIFRK

SEQ ID NO: 3 - protein, 241 aa, Dengue virus
ADLSLEKAAEVSWEEEAEHSGASHNILVEVQDDGTMKIKDEERDDTGGGGSGGGGSGVLWDTPSPPEVERAVLDDGIYRIMQRGLLGRSQVGVGVFQDGVFHTMWHVTRGAVLMYQGKRLEPSWASVKKDLISYGGGWRFQGSWNTGEEVQVIAVEPGKNPKNVQTAPGTFKTPEGEVGAIALDFKPGTSGSPIVNREGKIVGLYGNGVVTTSGTYVSAIAQAKASQEGPLPEIEDEVFRK

SEQ ID NO: 4 - protein, 237 aa, Dengue virus
DLTVEKAADVTWEEEAEQTGVSHNLMITVDDDGTMRIKDDETENILGGGGSGGGGSGVLWDVPSPPETQKAELEEGVYRIKQQGIFGKTQVGVGVQKEGVFHTMWHVTRGAVLTHNGKRLEPNWASVKKDLISYGGGWRLSAQWQKGEEVQVIAVEPGKNPKNFQTMPGIFQTTTGEIGAIALDFKPGTSGSPIINREGKVVGLYGNGVVTKNGGYVSGIAQTNAEPDGPTPELEEE

SEQ ID NO: 5 - protein, 241 aa, Dengue virus
ADLSLEKAANVQWDEMADITGSSPIIEVKQDEDGSFSIRDVEETNMIGGGGSGGGGSGALWDVPSPAAAQKATLTEGVYRIMQRGLFGKTQVGVGIHMEGVFHTMWHVTRGSVICHESGRLEPSWADVRNDMISYGGGWRLGDKWDKEEDVQVLAIEPGKNPKHVQTKPGLFKTLTGEIGAVTLDFKPGTSGSPIINKKGKVIGLYGNGVVTKSGDYVSAITQAERIGEPDYEVDEDIFRK

SEQ ID NO: 6 - protein, 7 aa, West Nile virus
MHHHHHH

SEQ ID NO: 7 - protein, 9 aa, West Nile virus
GGGGSGGGG